European Patent Application EP 4 454 662 A1, published October 30, 2024. Title: ANTI-DLL3 ANTIBODY AND PHARMACEUTICAL USE THEREOF, AND ANTIBODY-DRUG CONJUGATE CONTAINING ANTI-DLL3 ANTIBODY. Applicant: JIANGSU HENGRUI PHARMACEUTICALS CO., LTD. The sequence listing filed with the application follows.

SEQUENCE LISTING (65 sequences)

SEQ ID NO: 1 - protein, 618 aa, Homo sapiens
MVSPRMSGLLSQTVILALIFLPQTRPAGVFELQIHSFGPGPGPGAPRSPCSARLPCRLFFRVCLKPGLSEEAAESPCALGAALSARGPVYTEQPGAPAPDLPLPDGLLQVPFRDAWPGTFSFIIETWREELGDQIGGPAWSLLARVAGRRRLAAGGPWARDIQRAGAWELRFSYRARCEPPAVGTACTRLCRPRSAPSRCGPGLRPCAPLEDECEAPLVCRAGCSPEHGFCEQPGECRCLEGWTGPLCTVPVSTSSCLSPRGPSSATTGCLVPGPGPCDGNPCANGGSCSETPRSFECTCPRGFYGLRCEVSGVTCADGPCFNGGLCVGGADPDSAYICHCPPGFQGSNCEKRVDRCSLQPCRNGGLCLDLGHALRCRCRAGFAGPRCEHDLDDCAGRACANGGTCVEGGGAHRCSCALGFGGRDCRERADPCAARPCAHGGRCYAHFSGLVCACAPGYMGARCEFPVHPDGASALPAAPPGLRPGDPQRYLLPPALGLLVAAGVAGAALLLVHVRRRGHSQDAGSRLLAGTPEPSVHALPDALNNLRTQEGSGDGPSSSVDWNRPEDVDPQGIYVISAPSIYAREVATPLFPPLHTGRAGQRQHLLFPYPSSILSVK

SEQ ID NO: 2 - protein, 618 aa, Macaca fascicularis
MVSPRMSRLLSQTVILALIFIPQARPAGVFELQIHSFGPGPGPGAPRSPCSARGPCRLFFRVCLKPGLSEEAAESPCALGAALSARGPVYTEQPEAPAPDLPLPNGLLQVPFRDAWPGTFSLIIETWREELGDQIGGPAWSLLARVTRRRRLAAGGPWARDIQRAGAWELRFSYRARCELPAVGTACTRLCRPRSAPSRCGPGLRPCAPLEDECEAPPVCRAGCSLEHGFCEQPGECRCLEGWTGPLCMVPVSTSSCLGLRGPSSTTTGCLVPGPGPCDGNPCANGGSCSETPGSFECTCPRGFYGLRCEVSGVTCADGPCFNGGLCVGGADPDSAYICHCPPGFQGSNCEKRVDRCSLQPCRNGGLCLDLGHALRCRCRAGFAGPRCEHDLDDCAGRACANGGTCVEGGGAHRCSCALGFGGRNCRERADPCAARPCAHGGRCYAHFSGLVCACAPGYMGARCEFPVHPDGVSALPAAPPGLRPGDPQRYLLPPALGLLVAAGVAGAALLLVHVRRRGHAQDAGSRLLAGTPEPSVHALPDALNNLRTQEGPGDVPSSSVDWNRPEDVDSRGIYVISAPSIYAREVAMPLFPPLHTGRAGQRQNLLFPFPSSILSVK

SEQ ID NO: 3 - protein, 589 aa, Rattus norvegicus
MVSLQVSSLPQTLILAFLLPQALPAGVFELQIHSFGPGPGPGTPRSPCNARGPCRLFFRVCLKPGVSQEAAESLCALGAALSTSGPVYTEQPGVPAAALSLPDGLVRVPFLDAWPGTFSLIIETWREQLGERAAGPAWNLLARVAGRRRLAAGAPWARDVQRTGAWELHFSYRARCEPPAVGAACARLCRSRSAPSRCGPGLRPCTPFPDECEAPRESLTVCRAGCSPEHGYCEEPDECHCLEGWTGPLCTVPVSTSSCLNSRVSGPAGTGCLLPGPGPCDGNPCANGGSCSETPGSFECACPRGFYGPRCEVSGVTCADGPCFNGGLCVGGEDPDSAYVCHCPPAFQGSNCERRVDRCSLQPCQNGGLCLDLGHALRCRCRAGFAGPRCEHDLDDCAGRACANGGTCVEGGGARRCSCALGFGGRDCRERADPCASRPCAHGGRCYAHFSGLVCACAPGYMGVRCEFAVRPDGADAVPAAPRGLRQADSQRFLLPPALGLLAAAALAGAALLLIHVRRRGPGRDTGTRLLSGTREPSVHTLPDALNNLRLQDGAGDGPTSSADWNHPEDGDSRSIYVIPAPSIYAREA

SEQ ID NO: 4 - protein, 592 aa, Mus musculus
MVSLQVSPLSQTLILAFLLPQALPAGVFELQIHSFGPGPGLGTPRSPCNARGPCRLFFRVCLKPGVSQEATESLCALGAALSTSVPVYTEHPGESAAALPLPDGLVRVPFRDAWPGTFSLVIETWREQLGEHAGGPAWNLLARVVGRRRLAAGGPWARDVQRTGTWELHFSYRARCEPPAVGAACARLCRSRSAPSRCGPGLRPCTPFPDECEAPSVCRPGCSPEHGYCEEPDECRCLEGWTGPLCTVPVSTSSCLNSRVPGPASTGCLLPGPGPCDGNPCANGGSCSETSGSFECACPRGFYGLRCEVSGVTCADGPCFNGGLCVGGEDPDSAYVCHCPPGFQGSNCEKRVDRCSLQPCQNGGLCLDLGHALRCRCRAGFAGPRCEHDLDDCAGRACANGGTCVEGGGSRRCSCALGFGGRDCRERADPCASRPCAHGGRCYAHFSGLVCACAPGYMGVRCEFAVRPDGADAVPAAPRGLRQADPQRFLLPPALGLLVAAGLAGAALLVIHVRRRGPGQDTGTRLLSGTREPSVHTLPDALNNLRLQDGAGDGPSSSADWNHPEDGDSRSIYVIPAPSIYAREDWLIQVLF

SEQ ID NO: 5 - protein, 723 aa, Homo sapiens
MGSRCALALAVLSALLCQVWSSGVFELKLQEFVNKKGLLGNRNCCRGGAGPPPCACRTFFRVCLKHYQASVSPEPPCTYGSAVTPVLGVDSFSLPDGGGADSAFSNPIRFPFGFTWPGTFSLIIEALHTDSPDDLATENPERLISRLATQRHLTVGEEWSQDLHSSGRTDLKYSYRFVCDEHYYGEGCSVFCRPRDDAFGHFTCGERGEKVCNPGWKGPYCTEPICLPGCDEQHGFCDKPGECKCRVGWQGRYCDECIRYPGCLHGTCQQPWQCNCQEGWGGLFCNQDLNYCTHHKPCKNGATCTNTGQGSYTCSCRPGYTGATCELGIDECDPSPCKNGGSCTDLENSYSCTCPPGFYGKICELSAMTCADGPCFNGGRCSDSPDGGYSCRCPVGYSGFNCEKKIDYCSSSPCSNGAKCVDLGDAYLCRCQAGFSGRHCDDNVDDCASSPCANGGTCRDGVNDFSCTCPPGYTGRNCSAPVSRCEHAPCHNGATCHERGHRYVCECARGYGGPNCQFLLPELPPGPAVVDLTEKLEGQGGPFPWVAVCAGVILVLMLLLGCAAVVVCVRLRLQKHRPPADPCRGETETMNNLANCQREKDISVSIIGATQIKNTNKKADFHGDHSADKNGFKARYPAVDYNLVQDLKGDDTAVRDAHSKRDTKCQPQGSSGEEKGTPTTLRGGEASERKRPDSGCSTSKDTKYQSVYVISEEKDECVIATEV

SEQ ID NO: 6 - protein, 685 aa, Homo sapiens
MAAASRSASGWALLLLVALWQQRAAGSGVFQLQLQEFINERGVLASGRPCEPGCRTFFRVCLKHFQAVVSPGPCTFGTVSTPVLGTNSFAVRDDSSGGGRNPLQLPFNFTWPGTFSLIIEAWHAPGDDLRPEALPPDALISKIAIQGSLAVGQNWLLDEQTSTLTRLRYSYRVICSDNYYGDNCSRLCKKRNDHFGHYVCQPDGNLSCLPGWTGEYCQQPICLSGCHEQNGYCSKPAECLCRPGWQGRLCNECIPHNGCRHGTCSTPWQCTCDEGWGGLFCDQDLNYCTHHSPCKNGATCSNSGQRSYTCTCRPGYTGVDCELELSECDSNPCRNGGSCKDQEDGYHCLCPPGYYGLHCEHSTLSCADSPCFNGGSCRERNQGANYACECPPNFTGSNCEKKVDRCTSNPCANGGQCLNRGPSRMCRCRPGFTGTYCELHVSDCARNPCAHGGTCHDLENGLMCTCPAGFSGRRCEVRTSIDACASSPCFNRATCYTDLSTDTFVCNCPYGFVGSRCEFPVGLPPSFPWVAVSLGVGLAVLLVLLGMVAVAVRQLRLRRPDDGSREAMNNLSDFQKDNLIPAAQLKNTNQKKELEVDCGLDKSNCGKQQNHTLDYNLAPGPLGRGTMPGKFPHSDKSLGEKAPLRLHSEKPECRISAICSPRDSMYQSVCLISEERNECVIATEV

SEQ ID NO: 7 - protein, 507 aa, synthetic construct
  REGION 1..507: note = His-hDLL3(ECD)
METDTLLLWVLLLWVPGSTGHHHHHHHHHHGGGGGSGGGGSAGVFELQIHSFGPGPGPGAPRSPCSARLPCRLFFRVCLKPGLSEEAAESPCALGAALSARGPVYTEQPGAPAPDLPLPDGLLQVPFRDAWPGTFSFIIETWREELGDQIGGPAWSLLARVAGRRRLAAGGPWARDIQRAGAWELRFSYRARCEPPAVGTACTRLCRPRSAPSRCGPGLRPCAPLEDECEAPLVCRAGCSPEHGFCEQPGECRCLEGWTGPLCTVPVSTSSCLSPRGPSSATTGCLVPGPGPCDGNPCANGGSCSETPRSFECTCPRGFYGLRCEVSGVTCADGPCFNGGLCVGGADPDSAYICHCPPGFQGSNCEKRVDRCSLQPCRNGGLCLDLGHALRCRCRAGFAGPRCEHDLDDCAGRACANGGTCVEGGGAHRCSCALGFGGRDCRERADPCAARPCAHGGRCYAHFSGLVCACAPGYMGARCEFPVHPDGASALPAAPPGLRPGDPQRYL

SEQ ID NO: 8 - protein, 727 aa, synthetic construct
  REGION 1..727: note = Fc-hDLL3(ECD)
METDTLLLWVLLLWVPGSTGEPKSSDKTHTCPPCPAPELLGGPSVFLFPPKPKDTLMISRTPEVTCVVVDVSHEDPEVKFNWYVDGVEVHNAKTKPREEQYNSTYRVVSVLTVLHQDWLNGKEYKCKVSNKALPAPIEKTISKAKGQPREPQVYTLPPSRDELTKNQVSLTCLVKGFYPSDIAVEWESNGQPENNYKTTPPVLDSDGSFFLYSKLTVDKSRWQQGNVFSCSVMHEALHNHYTQKSLSLSPGGGGGSGGGGSAGVFELQIHSFGPGPGPGAPRSPCSARLPCRLFFRVCLKPGLSEEAAESPCALGAALSARGPVYTEQPGAPAPDLPLPDGLLQVPFRDAWPGTFSFIIETWREELGDQIGGPAWSLLARVAGRRRLAAGGPWARDIQRAGAWELRFSYRARCEPPAVGTACTRLCRPRSAPSRCGPGLRPCAPLEDECEAPLVCRAGCSPEHGFCEQPGECRCLEGWTGPLCTVPVSTSSCLSPRGPSSATTGCLVPGPGPCDGNPCANGGSCSETPRSFECTCPRGFYGLRCEVSGVTCADGPCFNGGLCVGGADPDSAYICHCPPGFQGSNCEKRVDRCSLQPCRNGGLCLDLGHALRCRCRAGFAGPRCEHDLDDCAGRACANGGTCVEGGGAHRCSCALGFGGRDCRERADPCAARPCAHGGRCYAHFSGLVCACAPGYMGARCEFPVHPDGASALPAAPPGLRPGDPQRYL

SEQ ID NO: 9 - protein, 514 aa, synthetic construct
  REGION 1..514: note = hDLL3(ECD)-strep twin
METDTLLLWVLLLWVPGSTGAGVFELQIHSFGPGPGPGAPRSPCSARLPCRLFFRVCLKPGLSEEAAESPCALGAALSARGPVYTEQPGAPAPDLPLPDGLLQVPFRDAWPGTFSFIIETWREELGDQIGGPAWSLLARVAGRRRLAAGGPWARDIQRAGAWELRFSYRARCEPPAVGTACTRLCRPRSAPSRCGPGLRPCAPLEDECEAPLVCRAGCSPEHGFCEQPGECRCLEGWTGPLCTVPVSTSSCLSPRGPSSATTGCLVPGPGPCDGNPCANGGSCSETPRSFECTCPRGFYGLRCEVSGVTCADGPCFNGGLCVGGADPDSAYICHCPPGFQGSNCEKRVDRCSLQPCRNGGLCLDLGHALRCRCRAGFAGPRCEHDLDDCAGRACANGGTCVEGGGAHRCSCALGFGGRDCRERADPCAARPCAHGGRCYAHFSGLVCACAPGYMGARCEFPVHPDGASALPAAPPGLRPGDPQRYLWSHPQFEKGGGSGGGSGGSAWSHPQFEK

SEQ ID NO: 10 - protein, 514 aa, synthetic construct
  REGION 1..514: note = cynoDLL3(ECD)-strep twin
METDTLLLWVLLLWVPGSTGAGVFELQIHSFGPGPGPGAPRSPCSARGPCRLFFRVCLKPGLSEEAAESPCALGAALSARGPVYTEQPEAPAPDLPLPNGLLQVPFRDAWPGTFSLIIETWREELGDQIGGPAWSLLARVTRRRRLAAGGPWARDIQRAGAWELRFSYRARCELPAVGTACTRLCRPRSAPSRCGPGLRPCAPLEDECEAPPVCRAGCSLEHGFCEQPGECRCLEGWTGPLCMVPVSTSSCLGLRGPSSTTTGCLVPGPGPCDGNPCANGGSCSETPGSFECTCPRGFYGLRCEVSGVTCADGPCFNGGLCVGGADPDSAYICHCPPGFQGSNCEKRVDRCSLQPCRNGGLCLDLGHALRCRCRAGFAGPRCEHDLDDCAGRACANGGTCVEGGGAHRCSCALGFGGRNCRERADPCAARPCAHGGRCYAHFSGLVCACAPGYMGARCEFPVHPDGVSALPAAPPGLRPGDPQRYLWSHPQFEKGGGSGGGSGGSAWSHPQFEK

SEQ ID NO: 11 - protein, 514 aa, synthetic construct
  REGION 1..514: note = mouDLL3(ECD)-strep twin
METDTLLLWVLLLWVPGSTGAGVFELQIHSFGPGPGLGTPRSPCNARGPCRLFFRVCLKPGVSQEATESLCALGAALSTSVPVYTEHPGESAAALPLPDGLVRVPFRDAWPGTFSLVIETWREQLGEHAGGPAWNLLARVVGRRRLAAGGPWARDVQRTGTWELHFSYRARCEPPAVGAACARLCRSRSAPSRCGPGLRPCTPFPDECEAPSVCRPGCSPEHGYCEEPDECRCLEGWTGPLCTVPVSTSSCLNSRVPGPASTGCLLPGPGPCDGNPCANGGSCSETSGSFECACPRGFYGLRCEVSGVTCADGPCFNGGLCVGGEDPDSAYVCHCPPGFQGSNCEKRVDRCSLQPCQNGGLCLDLGHALRCRCRAGFAGPRCEHDLDDCAGRACANGGTCVEGGGSRRCSCALGFGGRDCRERADPCASRPCAHGGRCYAHFSGLVCACAPGYMGVRCEFAVRPDGADAVPAAPRGLRQADPQRFLWSHPQFEKGGGSGGGSGGSAWSHPQFEK

SEQ ID NO: 12 - protein, 120 aa, Mus musculus
EVQLQQSGPVLVKPGASVKMSCKASGYTFTDYYMNWVKQSHGKSLEWIGIINPYSGVTIYNHKFKGKATLTVDKSSNTAYMELNSLTSEDSAVYYCARQDSLLDYAMDYWGQGTSVTVSS

SEQ ID NO: 13 - protein, 107 aa, Mus musculus
DILMTQSPSSMSVSLGDTVSITCHASQGISGNMGWLQQKPGKSFKGLIYHGANLEDGVPSRFSGSGSGADYSLTISSLESEDFADYYCVQYAQFPYTFGGGTKLEIK

SEQ ID NO: 14 - protein, 123 aa, Mus musculus
EVQLVESGGGLVKPGGSLKLSCAASGFTFSDSGMHWIRQAPEKGLEWVAYISSGSSTIHYADTVKGRFTISRDNAKNTLFLQMTSLRSEDTAMYYCASPLYYYGRSYNAVAYWGQGTSVTVSS

SEQ ID NO: 15 - protein, 107 aa, Mus musculus
DIQMNQSPSSLSASLGDTITITCHASQNINVWLSWYQQKPGNIPKLLIYKASDLHTGVPSRFSGSGSGTGFTLTISSLQPEDIATYYCQQGQSYPLTFGGGTKLEIK

SEQ ID NO: 16 - protein, 5 aa, Mus musculus
DYYMN

SEQ ID NO: 17 - protein, 17 aa, Mus musculus
IINPYSGVTIYNHKFKG

SEQ ID NO: 18 - protein, 11 aa, Mus musculus
QDSLLDYAMDY

SEQ ID NO: 19 - protein, 11 aa, Mus musculus
HASQGISGNMG

SEQ ID NO: 20 - protein, 7 aa, Mus musculus
HGANLED

SEQ ID NO: 21 - protein, 9 aa, Mus musculus
VQYAQFPYT

SEQ ID NO: 22 - protein, 5 aa, Mus musculus
DSGMH

SEQ ID NO: 23 - protein, 17 aa, Mus musculus
YISSGSSTIHYADTVKG

SEQ ID NO: 24 - protein, 14 aa, Mus musculus
PLYYYGRSYNAVAY

SEQ ID NO: 25 - protein, 11 aa, Mus musculus
HASQNINVWLS

SEQ ID NO: 26 - protein, 7 aa, Mus musculus
KASDLHT

SEQ ID NO: 27 - protein, 9 aa, Mus musculus
QQGQSYPLT

SEQ ID NO: 28 - protein, 330 aa, Homo sapiens [sequence omitted]

SEQ ID NO: 29 - protein, 107 aa, Homo sapiens [sequence omitted]

SEQ ID NO: 30 - protein, 14 aa, synthetic construct
  REGION 1..14: note = mAb100 HCDR3 1
PLYHYGRSYNAVAY

SEQ ID NO: 31 - protein, 14 aa, synthetic construct
  REGION 1..14: note = mAb100 HCDR3 2
PLYYYGRSYNGVAY

SEQ ID NO: 32 - protein, 120 aa, synthetic construct
  REGION 1..120: note = hAb6 VH1
EVQLVQSGAEVKKPGASVKVSCKASGYTFTDYYMNWVRQAPGQRLEWMGIINPYSGVTIYNHKFKGRVTITVDKSASTAYMELSSLRSEDTAVYYCARQDSLLDYAMDYWGQGTTVTVSS

SEQ ID NO: 33 - protein, 120 aa, synthetic construct
  REGION 1..120: note = hAb6 VH2
EVQLVQSGAEVKKPGASVKVSCKASGYTFTDYYMNWVRQAPGQRLEWMGIINPYSGVTIYNHKFKGRVTLTVDKSANTAYMELSSLRSEDTAVYYCARQDSLLDYAMDYWGQGTTVTVSS

SEQ ID NO: 34 - protein, 120 aa, synthetic construct
  REGION 1..120: note = hAb6 VH3
EVQLVQSGAEVKKPGASVKVSCKASGYTFTDYYMNWVRQAPGQRLEWIGIINPYSGVTIYNHKFKGRATLTVDKSANTAYMELSSLRSEDTAVYYCARQDSLLDYAMDYWGQGTTVTVSS

SEQ ID NO: 35 - protein, 120 aa, synthetic construct
  REGION 1..120: note = hAb6 VH4
EVQLVQSGAEVKKPGASVKVSCKASGYTFTDYYMNWVRQAPGKRLEWMGIINPYSGVTIYNHKFKGRVTLTVDKSANTAYMELSSLRSEDTAVYYCARQDSLLDYAMDYWGQGTTVTVSS

SEQ ID NO: 36 - protein, 120 aa, synthetic construct
  REGION 1..120: note = hAb6 VH5
EVQLVQSGSELKKPGASVKVSCKASGYTFTDYYMNWVRQAPGQGLEWMGIINPYSGVTIYNHKFKGRFVLSVDKSVSTAYLQISSLKAEDTAVYYCARQDSLLDYAMDYWGQGTTVTVSS

SEQ ID NO: 37 - protein, 120 aa, synthetic construct
  REGION 1..120: note = hAb6 VH6
EVQLVQSGSELKKPGASVKVSCKASGYTFTDYYMNWVRQAPGQGLEWMGIINPYSGVTIYNHKFKGRFVLSVDKSSNTAYLQISSLKAEDTAVYYCARQDSLLDYAMDYWGQGTTVTVSS

SEQ ID NO: 38 - protein, 120 aa, synthetic construct
  REGION 1..120: note = hAb6 VH7
EVQLVESGGGLVQPGGSLKLSCAASGYTFTDYYMNWVRQASGKGLEWVGIINPYSGVTIYNHKFKGRFTLSVDKSKNTAYLQMNSLKTEDTAVYYCARQDSLLDYAMDYWGQGTTVTVSS

SEQ ID NO: 39 - protein, 120 aa, synthetic construct
  REGION 1..120: note = hAb6VH8
QVQLVQSGAEVKKPGASVKVSCKASGYTFTDYYMNWVRQAPGQRLEWMGIINPYSGVTIYNHKFKGRVTITRDTSASTAYMELSSLRSEDTAVYYCARQDSLLDYAMDYWGQGTTVTVSS

SEQ ID NO: 40 - protein, 120 aa, synthetic construct
  REGION 1..120: note = hAb6VH9
QVQLVQSGSELKKPGASVKVSCKASGYTFTDYYMNWVRQAPGQGLEWMGIINPYSGVTIYNHKFKGRFVFSLDTSVSTAYLQISSLKAEDTAVYYCARQDSLLDYAMDYWGQGTTVTVSS

SEQ ID NO: 41 - protein, 120 aa, synthetic construct
  REGION 1..120: note = hAb6VH10
EVQLVESGGGLVQPGGSLKLSCAASGFTFSDYYMNWVRQASGKGLEWVGIINPYSGVTIYNHKFKGRFTISRDDSKNTAYLQMNSLKTEDTAVYYCTRQDSLLDYAMDYWGQGTTVTVSS

SEQ ID NO: 42 - protein, 120 aa, synthetic construct
  REGION 1..120: note = hAb6VH11
EVQLVQSGSELKKPGASVKVSCKASGYTFTDYYMNWVKQAPGQGLEWMGIINPYSGVTIYNHKFKGRFVLSVDKSSNTAYLQISSLKAEDTAVYYCARQDSLLDYAMDYWGQGTTVTVSS

SEQ ID NO: 43 - protein, 120 aa, synthetic construct
  REGION 1..120: note = hAb6VH12
EVQLVQSGSELKKPGASVKVSCKASGYTFTDYYMNWVRQAPGQGLEWMGIINPYSGVTIYNHKFKGRFALSVDKSSNTAYLQISSLKAEDTAVYYCARQDSLLDYAMDYWGQGTTVTVSS

SEQ ID NO: 44 - protein, 120 aa, synthetic construct
  REGION 1..120: note = hAb6VH13
EVQLVQSGSELKKPGASVKVSCKASGYTFTDYYMNWVKQAPGQGLEWMGIINPYSGVTIYNHKFKGRFALSVDKSSNTAYLQISSLKAEDTAVYYCARQDSLLDYAMDYWGQGTTVTVSS

SEQ ID NO: 45 - protein, 107 aa, synthetic construct
  REGION 1..107: note = hAb6 VL1
DIQMTQSPSSLSASVGDRVTITCHASQGISGNMGWLQQKPGKAPKGLIYHGANLEDGVPSRFSGSGSGTDFTLTISSLQPEDFATYYCVQYAQFPYTFGGGTKVEIK

SEQ ID NO: 46 - protein, 107 aa, synthetic construct
  REGION 1..107: note = hAb6 VL2
DIQMTQSPSSLSASVGDRVTITCHASQGISGNMGWLQQKPGKAPKGLIYHGANLEDGVPSRFSGSGSGADYTLTISSLQPEDFATYYCVQYAQFPYTFGGGTKVEIK

SEQ ID NO: 47 - protein, 107 aa, synthetic construct
  REGION 1..107: note = hAb6 VL3
DIQMTQSPSSLSASVGDRVTITCHASQGISGNMGWLQQKPGKSFKGLIYHGANLEDGVPSRFSGSGSGADYTLTISSLQPEDFATYYCVQYAQFPYTFGGGTKVEIK

SEQ ID NO: 48 - protein, 107 aa, synthetic construct
  REGION 1..107: note = hAb6 VL4
DIQMTQSPSSLSASVGDRVTITCHASQGISGNMGWLQQKPGKAPKGLIYHGANLEDGVPSRFSGSGSGADYTLTISSLQPEDFADYYCVQYAQFPYTFGGGTKVEIK

SEQ ID NO: 49 - protein, 107 aa, synthetic construct
  REGION 1..107: note = hAb6VL5
DIQMTQSPSSLSASVGDRVTITCHASQGISGNMGWFQQKPGKAPKSLIYHGANLEDGVPSRFSGSGSGTDFTLTISSLQPEDFATYYCVQYAQFPYTFGGGTKVEIK

SEQ ID NO: 50 - protein, 123 aa, synthetic construct
  REGION 1..123: note = hAb100 VH1
EVQLVESGGGLVKPGGSLRLSCAASGFTFSDSGMHWIRQAPGKGLEWVSYISSGSSTIHYADTVKGRFTISRDNAKNSLYLQMNSLRAEDTAVYYCASPLYYYGRSYNAVAYWGQGTTVTVSS

SEQ ID NO: 51 - protein, 123 aa, synthetic construct
  REGION 1..123: note = hAb100 VH2
EVQLVESGGGLVKPGGSLRLSCAASGFTFSDSGMHWIRQAPGKGLEWVAYISSGSSTIHYADTVKGRFTISRDNAKNSLYLQMNSLRAEDTAVYYCASPLYYYGRSYNAVAYWGQGTTVTVSS

SEQ ID NO: 52 - protein, 123 aa, synthetic construct
  REGION 1..123: note = hAb100 VH3
EVQLVESGGGLVKPGGSLRLSCAASGFTFSDSGMHWIRQAPGKGLEWVAYISSGSSTIHYADTVKGRFTISRDNAKNSLYLQMNSLRAEDTAVYYCASPLYHYGRSYNAVAYWGQGTTVTVSS

SEQ ID NO: 53 - protein, 123 aa, synthetic construct
  REGION 1..123: note = hAb100 VH4
EVQLVESGGGLVKPGGSLRLSCAASGFTFSDSGMHWIRQAPGKGLEWVAYISSGSSTIHYADTVKGRFTISRDNAKNSLYLQMNSLRAEDTAVYYCASPLYYYGRSYNGVAYWGQGTTVTVSS

SEQ ID NO: 54 - protein, 123 aa, synthetic construct
  REGION 1..123: note = hAb100VH5
QVQLVESGGGLVKPGGSLRLSCAASGFTFSDSGMHWIRQAPGKGLEWVSYISSGSSTIHYADTVKGRFTISRDNAKNSLYLQMNSLRAEDTAVYYCARPLYYYGRSYNAVAYWGQGTTVTVSS

SEQ ID NO: 55 - protein, 107 aa, synthetic construct
  REGION 1..107: note = hAb100 VL1
DIQMTQSPSSLSASVGDRVTITCHASQNINVWLSWYQQKPGKVPKLLIYKASDLHTGVPSRFSGSGSGTDFTLTISSLQPEDVATYYCQQGQSYPLTFGGGTKVEIK

SEQ ID NO: 56 - protein, 107 aa, synthetic construct
  REGION 1..107: note = hAb100 VL2
DIQMTQSPSSLSASVGDRVTITCHASQNINVWLSWYQQKPGKIPKLLIYKASDLHTGVPSRFSGSGSGTDFTLTISSLQPEDVATYYCQQGQSYPLTFGGGTKVEIK

SEQ ID NO: 57 - protein, 14 aa, synthetic construct
  REGION 1..14: note = hAb100 HCDR3
  VARIANT 4: note = Xaa is Y or H
  VARIANT 11: note = Xaa is A or G
PLYXYGRSYNXVAY

SEQ ID NO: 58 - protein, 450 aa, synthetic construct
  REGION 1..450: note = Hu6
EVQLVQSGSELKKPGASVKVSCKASGYTFTDYYMNWVRQAPGQGLEWMGIINPYSGVTIYNHKFKGRFALSVDKSSNTAYLQISSLKAEDTAVYYCARQDSLLDYAMDYWGQGTTVTVSSASTKGPSVFPLAPSSKSTSGGTAALGCLVKDYFPEPVTVSWNSGALTSGVHTFPAVLQSSGLYSLSSVVTVPSSSLGTQTYICNVNHKPSNTKVDKKVEPKSCDKTHTCPPCPAPELLGGPSVFLFPPKPKDTLMISRTPEVTCVVVDVSHEDPEVKFNWYVDGVEVHNAKTKPREEQYNSTYRVVSVLTVLHQDWLNGKEYKCKVSNKALPAPIEKTISKAKGQPREPQVYTLPPSRDELTKNQVSLTCLVKGFYPSDIAVEWESNGQPENNYKTTPPVLDSDGSFFLYSKLTVDKSRWQQGNVFSCSVMHEALHNHYTQKSLSLSPGK

SEQ ID NO: 59 - protein, 214 aa, synthetic construct
  REGION 1..214: note = Hu6
DIQMTQSPSSLSASVGDRVTITCHASQGISGNMGWLQQKPGKAPKGLIYHGANLEDGVPSRFSGSGSGADYTLTISSLQPEDFADYYCVQYAQFPYTFGGGTKVEIKRTVAAPSVFIFPPSDEQLKSGTASVVCLLNNFYPREAKVQWKVDNALQSGNSQESVTEQDSKDSTYSLSSTLTLSKADYEKHKVYACEVTHQGLSSPVTKSFNRGEC

SEQ ID NO: 60 - protein, 453 aa, synthetic construct
  REGION 1..453: note = Hu100
EVQLVESGGGLVKPGGSLRLSCAASGFTFSDSGMHWIRQAPGKGLEWVSYISSGSSTIHYADTVKGRFTISRDNAKNSLYLQMNSLRAEDTAVYYCASPLYYYGRSYNAVAYWGQGTTVTVSSASTKGPSVFPLAPSSKSTSGGTAALGCLVKDYFPEPVTVSWNSGALTSGVHTFPAVLQSSGLYSLSSVVTVPSSSLGTQTYICNVNHKPSNTKVDKKVEPKSCDKTHTCPPCPAPELLGGPSVFLFPPKPKDTLMISRTPEVTCVVVDVSHEDPEVKFNWYVDGVEVHNAKTKPREEQYNSTYRVVSVLTVLHQDWLNGKEYKCKVSNKALPAPIEKTISKAKGQPREPQVYTLPPSRDELTKNQVSLTCLVKGFYPSDIAVEWESNGQPENNYKTTPPVLDSDGSFFLYSKLTVDKSRWQQGNVFSCSVMHEALHNHYTQKSLSLSPGK

SEQ ID NO: 61 - protein, 214 aa, synthetic construct
  REGION 1..214: note = Hu100
DIQMTQSPSSLSASVGDRVTITCHASQNINVWLSWYQQKPGKVPKLLIYKASDLHTGVPSRFSGSGSGTDFTLTISSLQPEDVATYYCQQGQSYPLTFGGGTKVEIKRTVAAPSVFIFPPSDEQLKSGTASVVCLLNNFYPREAKVQWKVDNALQSGNSQESVTEQDSKDSTYSLSSTLTLSKADYEKHKVYACEVTHQGLSSPVTKSFNRGEC

SEQ ID NO: 62 - protein, 454 aa, synthetic construct
  REGION 1..454: note = BI-764532
QVQLVQSGAEVKKPGASVKVSCKASGYTFTSYYVHWVRQAPGQGLEWMVIINPGGGTTSYAQKFLGRVTMTRDTSTNTVYMELKSLRSEDTAVYYCARGEAVTGNYFYYGMDVWGQGTTVTVSSASTKGPSVFPLAPSSKSTSGGTAALGCLVKDYFPEPVTVSWNSGALTSGVHTFPAVLQSSGLYSLSSVVTVPSSSLGTQTYICNVNHKPSNTKVDKKVEPKSCDKTHTCPPCPAPELLGGPSVFLFPPKPKDTLMISRTPEVTCVVVDVSHEDPEVKFNWYVDGVEVHNAKTKPREEQYNSTYRVVSVLTVLHQDWLNGKEYKCKVSNKALPAPIEKTISKAKGQPREPQVYTLPPSRDELTKNQVSLTCLVKGFYPSDIAVEWESNGQPENNYKTTPPVLDSDGSFFLYSKLTVDKSRWQQGNVFSCSVMHEALHNHYTQKSLSLSPGK

SEQ ID NO: 63 - protein, 214 aa, synthetic construct
  REGION 1..214: note = BI-764532
DIQMTQSPSAMSASVGDRVTITCRASQGISNYLVWFQQKPGKAPKRLIYAVSSLYSGVPSRFSGSGSGTEFTLTISSLQPEDFATYYCLQHDSYPYTFGQGTKLEIKRTVAAPSVFIFPPSDEQLKSGTASVVCLLNNFYPREAKVQWKVDNALQSGNSQESVTEQDSKDSTYSLSSTLTLSKADYEKHKVYACEVTHQGLSSPVTKSFNRGEC

SEQ ID NO: 64 - protein, 448 aa, synthetic construct
  REGION 1..448: note = C25
QVQLVQSGAEVKKPGASVKVSCKASGYTFTNSWIGWFRQAPGQGLEWIGDIYPGGGYTNYNEIFKGKATMTADTSTNTAYMELSSLRSEDTAVYYCSRGIPGYAMDYWGQGTLVTVSSASTKGPSVFPLAPSSKSTSGGTAALGCLVKDYFPEPVTVSWNSGALTSGVHTFPAVLQSSGLYSLSSVVTVPSSSLGTQTYICNVNHKPSNTKVDKKVEPKSCDKTHTCPPCPAPELLGGPSVFLFPPKPKDTLMISRTPEVTCVVVDVSHEDPEVKFNWYVDGVEVHNAKTKPREEQYNSTYRVVSVLTVLHQDWLNGKEYKCKVSNKALPAPIEKTISKAKGQPREPQVYTLPPSRDELTKNQVSLTCLVKGFYPSDIAVEWESNGQPENNYKTTPPVLDSDGSFFLYSKLTVDKSRWQQGNVFSCSVMHEALHNHYTQKSLSLSPGK

SEQ ID NO: 65 - protein, 220 aa, synthetic construct
  REGION 1..220: note = C25
DIQMTQSPSSLSASVGDRVTMSCKSSQSLLNSGDQKNYLTWYQQKPGKAPKLLIYWASTGESGVPSRFSGSGSGTDFTFTISSLQPEDIATYYCQNDYSYPWTFGQGTKVEIKRTVAAPSVFIFPPSDEQLKSGTASVVCLLNNFYPREAKVQWKVDNALQSGNSQESVTEQDSKDSTYSLSSTLTLSKADYEKHKVYACEVTHQGLSSPVTKSFNRGEC